European Patent Application EP 4 678 241 A2, published January 14, 2026. Title: A QUADRICISTRONIC SYSTEM COMPRISING A HOMING RECEPTOR OR A CYTOKINE, AND CHIMERIC ANTIGEN RECEPTOR FOR GENETIC MODIFICATION OF IMMUNOTHERAPIES. Applicant: ImmunityBio, Inc. Application EP. The sequence listing filed with the application follows.

SEQUENCE LISTING (69 sequences)

SEQ ID NO: 1 - DNA, 1119 bp, synthetic construct
  misc_feature 1..1119: note = Laboratory made
  source 1..1119: mol_type = other DNA
atgaaaagcgtgctggtggtggctctccttgtcattttccaggtatgcctgtgtcaagatgaggtcacggacgattacatcggagacaacaccacagtggactacactttgttcgagtctttgtgctccaagaaggacgtgcggaactttaaagcctggttcctccctatcatgtactccatcatttgtttcgtgggcctactgggcaatgggctggtcgtgttgacctatatctatttcaagaggctcaagaccatgaccgatacctacctgctcaacctggcggtggcagacatcctcttcctcctgacccttcccttctgggcctacagcgcggccaagtcctgggtcttcggtgtccacttttgcaagctcatctttgccatctacaagatgagcttcttcagtggcatgctcctacttctttgcatcagcattgaccgctacgtggccatcgtccaggctgtctcagctcaccgccaccgtgcccgcgtccttctcatcagcaagctgtcctgtgtgggcatctggatactagccacagtgctctccatcccagagctcctgtacagtgacctccagaggagcagcagtgagcaagcgatgcgatgctctctcatcacagagcatgtggaggcctttatcaccatccaggtggcccagatggtgatcggctttctggtccccctgctggccatgagcttctgttaccttgtcatcatccgcaccctgctccaggcacgcaactttgagcgcaacaaggccatcaaggtgatcatcgctgtggtcgtggtcttcatagtcttccagctgccctacaatggggtggtcctggcccagacggtggccaacttcaacatcaccagtagcacctgtgagctcagtaagcaactcaacatcgcctacgacgtcacctacagcctggcctgcgtccgctgctgcgtcaaccctttcttgtacgccttcatcggcgtcaagttccgcaacgatctcttcaagctcttcaaggacctgggctgcctcagccaggagcagctccggcagtggtcttcctgtcggcacatccggcgctcctccatgagtgtggaggccgagaccaccaccaccttctccccatag

SEQ ID NO: 2 - DNA, 405 bp, synthetic construct
  misc_feature 1..405: note = Laboratory made
  source 1..405: mol_type = other DNA
atggctcagtcactggctctgagcctccttatcctggttctggcctttggcatccccaggacccaaggcagtgatggaggggctcaggactgttgcctcaagtacagccaaaggaagattcccgccaaggttgtccgcagctaccggaagcaggaaccaagcttaggctgctccatcccagctatcctgttcttgccccgcaagcgctctcaggcagagctatgtgcagacccaaaggagctctgggtgcagcagctgatgcagcatctggacaagacaccatccccacagaaaccagcccagggctgcaggaaggacaggggggcctccaagactggcaagaaaggaaagggctccaaaggctgcaagaggactgagcggtcacagacccctaaagggccatag

SEQ ID NO: 3 - DNA, 1178 bp, synthetic construct
  misc_feature 1..1178: note = laboratory made
  source 1..1178: mol_type = other DNA
gctccggtgcccgtcagtgggcagagcgcacatcgcccacagtccccgagaagttggggggaggggtcggcaattgaaccggtgcctagagaaggtggcgcggggtaaactgggaaagtgatgtcgtgtactggctccgcctttttcccgagggtgggggagaaccgtatataagtgcagtagtcgccgtgaacgttctttttcgcaacgggtttgccgccagaacacaggtaagtgccgtgtgtggttcccgcgggcctggcctctttacgggttatggcccttgcgtgccttgaattacttccacctggctgcagtacgtgattcttgatcccgagcttcgggttggaagtgggtgggagagttcgaggccttgcgcttaaggagccccttcgcctcgtgcttgagttgaggcctggcctgggcgctggggccgccgcgtgcgaatctggtggcaccttcgcgcctgtctcgctgctttcgataagtctctagccatttaaaatttttgatgacctgctgcgacgctttttttctggcaagatagtcttgtaaatgcgggccaagatctgcacactggtatttcggtttttggggccgcgggcggcgacggggcccgtgcgtcccagcgcacatgttcggcgaggcggggcctgcgagcgcggccaccgagaatcggacgggggtagtctcaagctggccggcctgctctggtgcctggcctcgcgccgccgtgtatcgccccgccctgggcggcaaggctggcccggtcggcaccagttgcgtgagcggaaagatggccgcttcccggccctgctgcagggagctcaaaatggaggacgcggcgctcgggagagcgggcgggtgagtcacccacacaaaggaaaagggcctttccgtcctcagccgtcgcttcatgtgactccacggagtaccgggcgccgtccaggcacctcgattagttctcgagcttttggagtacgtcgtctttaggttggggggaggggttttatgcgatggagtttccccacactgagtgggtggagactgaagttaggccagcttggcacttgatgtaattctccttggaatttgccctttttgagtttggatcttggttcattctcaagcctcagacagtggttcaaagtttttttcttccatttcaggtgtcgtga

SEQ ID NO: 4 - DNA, 30 bp, synthetic construct
  misc_feature 1..30: note = laboratory made
  source 1..30: mol_type = other DNA
ggaggaaaaactgtttcatacagaaggcgt

SEQ ID NO: 5 - DNA, 32 bp, synthetic construct
  misc_feature 1..32: note = laboratory made
  source 1..32: mol_type = other DNA
tagagggtatataatggaagctcgaattccag

SEQ ID NO: 6 - DNA, 320 bp, synthetic construct
  misc_feature 1..320: note = laboratory made
  source 1..320: mol_type = other DNA
aataaaatatctttattttcattacatctgtgtgttggttttttgtgtgaatcgatagtactaacatacgctctccatcaaaacaaaacgaaacaaaacaaactagcaaaataggctgtccccagtgcaagtgcaggtgccagaacatttctctggcctaactggccggtacctgagctcgctagcggaggaaaaactgtttcatacagaaggcgtggaggaaaaactgtttcatacagaaggcgtggaggaaaaactgtttcatacagaaggcgtagatctagactctagagggtatataatggaagctcgaattccag

SEQ ID NO: 7 - DNA, 6887 bp, synthetic construct
  misc_feature 1..6887: note = laboratory made
  source 1..6887: mol_type = other DNA
aggtcctgctttctctgacctgcattctctcccctgggcctgtgccgctttctgtctgcagcttgtggcctgggtcacctctacggctggcccagatccttccctgccgcctccttcaggttccgtcttcctccactccctcttccccttgctctctgctgtgttgctgcccaaggatgctctttccggagcacttccttctcggcgctgcaccacgtgatgtcctctgagcggatcctccccgtgtctgggtcctctccgggcatctctcctccctcacccaaccccatgccgtcttcactcgctgggttcccttttccttctccttctggggcctgtgccatctctcgtttcttaggatggccttctccgacggatgtctcccttgcgtcccgcctccccttcttgtaggcctgcatcatcaccgtttttctggacaaccccaaagtaccccgtctccctggctttagccacctctccatcctcttgctttctttgcctggacaccccgttctcctgtggattcgggtcacctctcactcctttcatttgggcagctcccctaccccccttacctctctagtctgtgctagctcttccagccccctgtcatggcatcttccaggggtccgagagctcagctagtcttcttcctccaacccgggcccctatgtccacttcaggacagcatgtttgctgcctccagggatcctgtgtccccgagctgggaccaccttatattcccagggccggttaatgtggctctggttctgggtacttttatctgtcccctccaccccacagtggggtacctctagagctgaccaaaagagcaccaaaggcgccctgaccttcagcccctacctgcgctccggtgcccgtcagtgggcagagcgcacatcgcccacagtccccgagaagttggggggaggggtcggcaattgaaccggtgcctagagaaggtggcgcggggtaaactgggaaagtgatgtcgtgtactggctccgcctttttcccgagggtgggggagaaccgtatataagtgcagtagtcgccgtgaacgttctttttcgcaacgggtttgccgccagaacacaggtaagtgccgtgtgtggttcccgcgggcctggcctctttacgggttatggcccttgcgtgccttgaattacttccacctggctgcagtacgtgattcttgatcccgagcttcgggttggaagtgggtgggagagttcgaggccttgcgcttaaggagccccttcgcctcgtgcttgagttgaggcctggcctgggcgctggggccgccgcgtgcgaatctggtggcaccttcgcgcctgtctcgctgctttcgataagtctctagccatttaaaatttttgatgacctgctgcgacgctttttttctggcaagatagtcttgtaaatgcgggccaagatctgcacactggtatttcggtttttggggccgcgggcggcgacggggcccgtgcgtcccagcgcacatgttcggcgaggcggggcctgcgagcgcggccaccgagaatcggacgggggtagtctcaagctggccggcctgctctggtgcctggcctcgcgccgccgtgtatcgccccgccctgggcggcaaggctggcccggtcggcaccagttgcgtgagcggaaagatggccgcttcccggccctgctgcagggagctcaaaatggaggacgcggcgctcgggagagcgggcgggtgagtcacccacacaaaggaaaagggcctttccgtcctcagccgtcgcttcatgtgactccacggagtaccgggcgccgtccaggcacctcgattagttctcgagcttttggagtacgtcgtctttaggttggggggaggggttttatgcgatggagtttccccacactgagtgggtggagactgaagttaggccagcttggcacttgatgtaattctccttggaatttgccctttttgagtttggatcttggttcattctcaagcctcagacagtggttcaaagtttttttcttccatttcaggtgtcgtgataatacgactcactatagggagacccaagctggaattcggcggccgccaccatgaaaagcgtgctggtggtggctctccttgtcattttccaggtatgcctgtgtcaagatgaggtcacggacgattacatcggagacaacaccacagtggactacactttgttcgagtctttgtgctccaagaaggacgtgcggaactttaaagcctggttcctccctatcatgtactccatcatttgtttcgtgggcctactgggcaatgggctggtcgtgttgacctatatctatttcaagaggctcaagaccatgaccgatacctacctgctcaacctggcggtggcagacatcctcttcctcctgacccttcccttctgggcctacagcgcggccaagtcctgggtcttcggtgtccacttttgcaagctcatctttgccatctacaagatgagcttcttcagtggcatgctcctacttctttgcatcagcattgaccgctacgtggccatcgtccaggctgtctcagctcaccgccaccgtgcccgcgtccttctcatcagcaagctgtcctgtgtgggcatctggatactagccacagtgctctccatcccagagctcctgtacagtgacctccagaggagcagcagtgagcaagcgatgcgatgctctctcatcacagagcatgtggaggcctttatcaccatccaggtggcccagatggtgatcggctttctggtccccctgctggccatgagcttctgttaccttgtcatcatccgcaccctgctccaggcacgcaactttgagcgcaacaaggccatcaaggtgatcatcgctgtggtcgtggtcttcatagtcttccagctgccctacaatggggtggtcctggcccagacggtggccaacttcaacatcaccagtagcacctgtgagctcagtaagcaactcaacatcgcctacgacgtcacctacagcctggcctgcgtccgctgctgcgtcaaccctttcttgtacgccttcatcggcgtcaagttccgcaacgatctcttcaagctcttcaaggacctgggctgcctcagccaggagcagctccggcagtggtcttcctgtcggcacatccggcgctcctccatgagtgtggaggccgagaccaccaccaccttctccccataggcggccgcggtcatagctgtttcctgaacagatcccgggtggcatccctgtgacccctccccagtgcctctcctggccctggaagttgccactccagtgcccaccagccttgtcctaataaaattaagttgcatcattttgtctgactaggtgtccttctataatattatggggtggaggggggtggtatggagcaaggggcaagttgggaagacaacctgtagggcctgcggggtctattgggaaccaagctggagtgcagtggcacaatcttggctcactgcaatctccgcctcctgggttcaagcgattctcctgcctcagcctcccgagttgttgggattccaggcatgcatgaccaggctcagctaatttttgtttttttggtagagacggggtttcaccatattggccaggctggtctccaactcctaatctcaggtgatctacccaccttggcctcccaaattgctgggattacaggcgtgaaccactgctcccttccctgtccttctgattttaaaataactataccagcaggaggacgtccagacacagcataggctacctggccatgcccaaccggtgggacatttgagttgcttgcttggcactgtcctctcatgcgttgggtccactcagtagatgcctgttgaattgggtacgcggccagcttaatgcataacttcgtataatgtatgctatacgaagttatgttaattaagggtgcagcggcctccgcgccgggttttggcgcctcccgcgggcgcccccctcctcacggcgagcgctgccacgtcagacgaagggcgcaggagcgttcctgatccttccgcccggacgctcaggacagcggcccgctgctcataagactcggccttagaaccccagtatcagcagaaggacattttaggacgggacttgggtgactctagggcactggttttctttccagagagcggaacaggcgaggaaaagtagtcccttctcggcgattctgcggagggatctccgtggggcggtgaacgccgatgattatataaggacgcgccgggtgtggcacagctagttccgtcgcagccgggatttgggtcgcggttcttgtttgtggatcgctgtgatcgtcacttggtgagttgcgggctgctgggctggccggggctttcgtggccgccgggccgctcggtgggacggaagcgtgtggagagaccgccaagggctgtagtctgggtccgcgagcaaggttgccctgaactgggggttggggggagcgcacaaaatggcggctgttcccgagtcttgaatggaagacgcttgtaaggcgggctgtgaggtcgttgaaacaaggtggggggcatggtgggcggcaagaacccaaggtcttgaggccttcgctaatgcgggaaagctcttattcgggtgagatgggctggggcaccatctggggaccctgacgtgaagtttgtcactgactggagaactcgggtttgtcgtctggttgcgggggcggcagttatgcggtgccgttgggcagtgcacccgtacctttgggagcgcgcgcctcgtcgtgtcgtgacgtcacccgttctgttggcttataatgcagggtggggccacctgccggtaggtgtgcggtaggcttttctccgtcgcaggacgcagggttcgggcctagggtaggctctcctgaatcgacaggcgccggacctctggtgaggggagggataagtgaggcgtcagtttctttggtcggttttatgtacctatcttcttaagtagctgaagctccggttttgaactatgcgctcggggttggcgagtgtgttttgtgaagttttttaggcaccttttgaaatgtaatcatttgggtcaatatgtaattttcagtgttagactagtaaattgtccgctaaattctggccgtttttggcttttttgttagacgaagcttgggctgcaggtcgactctagtgtaacgccaccatgaccgagtacaagcctaccgtgaggctggccacccgggacgacgtgcccagagccgtgaggacactggccgccgccttcgccgactaccccgccacccggcacaccgtggaccccgaccggcacatcgagcgggtgaccgagctgcaggaactgttcctgaccagagtgggcctggatatcggcaaagtgtgggtggccgacgacggagccgccgtggccgtgtggaccacccccgagtccgtggaggccggagccgtgtttgccgagatcggccccaggatggccgagctgtccggcagcaggctggccgcccagcagcagatggaaggcctgctggcccctcaccggcccaaagagcccgcctggttcctggccaccgtgggcgtgagccccgaccaccagggcaagggcctgggcagcgccgtggtgctgccaggcgtggaagccgccgagagggccggagtgcccgccttcctggaaaccagcgcccccaggaacctgcccttctacgagcggctgggctttaccgtgaccgccgacgtggaggtgccagagggccccaggacctggtgcatgacccggaagccaggcgcctgagaaaagcttataacttcgtataatgtatgctatacgaagttataacttgtttattgcagcttataatggttacaaataaagcaatagcatcacaaatttcacaaataaagcatttttttcactgcattctagttgtggtttgtccaaactcatcaatgtatcttatcatgtctgtgcggtgggctctatggcttctgaggcggaaagaaccagctggggctctagggggtatcccctctagagtactagggacaggattggtgacagaaaagccccatccttaggcctcctccttcctagtctcctgatattgggtctaacccccacctcctgttaggcagattccttatctggtgacacacccccatttcctggagccatctctctccttgccagaacctctaaggtttgcttacgatggagccagagaggatcctgggagggagagcttggcagggggtgggagggaagggggggatgcgtgacctgcccggttctcagtggccaccctgcgctaccctctcccagaacctgagctgctctgacgcggctgtctggtgcgtttcactgatcctggtgctgcagcttccttacacttcccaagaggagaagcagtttggaaaaacaaaatcagaataagttggtcctgagttctaactttggctcttcacctttctagtccccaatttatattgttcctccgtgcgtcagttttacctgtgagataaggccagtagccagccccgtcctggcagggctgtggtgaggaggggggtgtccgtgtggaaaactccctttgtgagaatggtgcgtcctaggtgttcaccaggtcgtggccgcctctactccctttctctttctccatccttctttccttaaagagtccccagtgctatctgggacatattcctccgcccagagcagggtcccgcttccctaaggccctgctctgggcttctgggtttgagtccttggcaagcccaggagaggcgctcaggcttccctgtcccccttcctcgtccaccatctcatgcccctggctctcctgccccttccctacaggggttcctggctctgctcttcagact

SEQ ID NO: 8 - DNA, 2497 bp, synthetic construct
  misc_feature 1..2497: note = laboratory made
  source 1..2497: mol_type = other DNA
ataacttcgtataatgtatgctatacgaagttatggcgcgccgaagttcctattcttctagaagaataggaacttccgaataggaacttcctgcacgtgaacttgtttattgcagcttataatggttacaaataaagcaatagcatcacaaatttcacaaataaagcatttttttcactgcattctagttgtggtttgtccaaactcatcaatgtatcttatcatgtctgtgagctgaaggtacgctgtatctcagtcagtcaagctagctcaggtttagttcctggtgtacttgagggggatgagttcctcaatggtggttttgaccagcttgccattcatctcaatgagcacaaagcagtcaggagcatagtcagagatcagctctctacacatgccacaggggctgaccaccctgatggatctgtccacctcatcagagtaggggtgcctgacagccacaatggtgtcaaagtccttctgcccgttgctcacagcagacccaatggcaatggcttcagcacagacagtgaccctgccaatgtaggcttcaatgtggacagcagagatgatctccccagtcttggtcctgatggccgccccgacatggtgcttgttgtcctcatagagcatggtgatcttctcagtggcgacctccaccagctccagatcctgctgagagatgttgaaggttttcatgttgggatccacgtggagctctgcttatatagacctcccaccgtacacgcctaccgcccatttgcgtcaacggggcggggttattacgacattttggaaagtcccgttgattttggtgccaaaacaaactcccattgacgtcaatggggtggagacttggaaatccccgtgagtcaaaccgctatccacgcccattggtgtactgccaaaaccgcatcaccatggtgaagttcctattctctagaaagaataggaacttccgaataggaacttcggtacgggaggtattggacaggccgcaataaaatatctttattttcattacatctgtgtgttggttttttgtgtgaatcgatagtactaacatacgctctccatcaaaacaaaacgaaacaaaacaaactagcaaaataggctgtccccagtgcaagtgcaggtgccagaacatttctctggcctaactggccggtacctgagctcgctagcggaggaaaaactgtttcatacagaaggcgtggaggaaaaactgtttcatacagaaggcgtggaggaaaaactgtttcatacagaaggcgtagatctagactctagagggtatataatggaagctcgaattccagcttggcattccggtactgttggtaaaaagcttggcaatccggtactgcctgcaggaccgccatggctcagtcactggctctgagcctccttatcctggttctggcctttggcatccccaggacccaaggcagtgatggaggggctcaggactgttgcctcaagtacagccaaaggaagattcccgccaaggttgtccgcagctaccggaagcaggaaccaagcttaggctgctccatcccagctatcctgttcttgccccgcaagcgctctcaggcagagctatgtgcagacccaaaggagctctgggtgcagcagctgatgcagcatctggacaagacaccatccccacagaaaccagcccagggctgcaggaaggacaggggggcctccaagactggcaagaaaggaaagggctccaaaggctgcaagaggactgagcggtcacagaccccttaagaattcgcggccgcggtcatagctgtttcctgaacagatcccgggtggcatccctgtgacccctccccagtgcctctcctggccctggaagttgccactccagtgcccaccagccttgtcctaataaaattaagttgcatcattttgtctgactaggtgtccttctataatattatggggtggaggggggtggtatggagcaaggggcaagttgggaagacaacctgtagggcctgcggggtctattgggaaccaagctggagtgcagtggcacaatcttggctcactgcaatctccgcctcctgggttcaagcgattctcctgcctcagcctcccgagttgttgggattccaggcatgcatgaccaggctcagctaatttttgtttttttggtagagacggggtttcaccatattggccaggctggtctccaactcctaatctcaggtgatctacccaccttggcctcccaaattgctgggattacaggcgtgaaccactgctcccttccctgtccttctgattttaaaataactataccagcaggaggacgtccagacacagcataggctacctggccatgcccaaccggtgggacatttgagttgcttgcttggcactgtcctctcatgcgttgggtccactcagtagatgcctgttgaattgggtacgcggccagcttaatgcataacttcgtataatgtatgctatacgaagttat

SEQ ID NO: 9 - DNA, 1211 bp, synthetic construct
  misc_feature 1..1211: note = laboratory made
  source 1..1211: mol_type = other DNA
ggcctccgcgccgggttttggcgcctcccgcgggcgcccccctcctcacggcgagcgctgccacgtcagacgaagggcgcaggagcgttcctgatccttccgcccggacgctcaggacagcggcccgctgctcataagactcggccttagaaccccagtatcagcagaaggacattttaggacgggacttgggtgactctagggcactggttttctttccagagagcggaacaggcgaggaaaagtagtcccttctcggcgattctgcggagggatctccgtggggcggtgaacgccgatgattatataaggacgcgccgggtgtggcacagctagttccgtcgcagccgggatttgggtcgcggttcttgtttgtggatcgctgtgatcgtcacttggtgagttgcgggctgctgggctggccggggctttcgtggccgccgggccgctcggtgggacggaagcgtgtggagagaccgccaagggctgtagtctgggtccgcgagcaaggttgccctgaactgggggttggggggagcgcacaaaatggcggctgttcccgagtcttgaatggaagacgcttgtaaggcgggctgtgaggtcgttgaaacaaggtggggggcatggtgggcggcaagaacccaaggtcttgaggccttcgctaatgcgggaaagctcttattcgggtgagatgggctggggcaccatctggggaccctgacgtgaagtttgtcactgactggagaactcgggtttgtcgtctggttgcgggggcggcagttatgcggtgccgttgggcagtgcacccgtacctttgggagcgcgcgcctcgtcgtgtcgtgacgtcacccgttctgttggcttataatgcagggtggggccacctgccggtaggtgtgcggtaggcttttctccgtcgcaggacgcagggttcgggcctagggtaggctctcctgaatcgacaggcgccggacctctggtgaggggagggataagtgaggcgtcagtttctttggtcggttttatgtacctatcttcttaagtagctgaagctccggttttgaactatgcgctcggggttggcgagtgtgttttgtgaagttttttaggcaccttttgaaatgtaatcatttgggtcaatatgtaattttcagtgttagactagtaaattgtccgctaaattctggccgtttttggcttttttgttagac

SEQ ID NO: 10 - DNA, 500 bp, synthetic construct
  misc_feature 1..500: note = laboratory made
  source 1..500: mol_type = other DNA
gggtaggggaggcgcttttcccaaggcagtctggagcatgcgctttagcagccccgctgggcacttggcgctacacaagtggcctctggcctcgcacacattccacatccaccggtaggcgccaaccggctccgttctttggtggccccttcgcgccaccttctacccctcccctagtcaggaagttcccccccgccccgcagctcgcgtcatgcaggacgtgacaaatggaagtagcacgtctcactagtctcgtgcaaatggacagcaccgctgagcaatggaagcgggtaggcccttggggcagcggccaatagcagctttgctccttcgctttctgggctcagaggctgggaaggggtgggtccgggggcgggctcaggggcgggctcaggggcggggcgggcgcccgaaggtcctccggaggcccggcattccgcacgcttcaaaagcgcacgtctgccgcgctgttctcttcttcctcatctccgggcctttcg

SEQ ID NO: 11 - DNA, 508 bp, synthetic construct
  misc_feature 1..508: note = laboratory made
  source 1..508: mol_type = other DNA
cgttacataacttacggtaaatggcccgcctggctgaccgcccaacgacccccgcccattgacgtcaataatgacgtatgttcccatagtaacgccaatagggactttccattgacgtcaatgggtggagtatttacggtaaactgcccacttggcagtacatcaagtgtatcatatgccaagtacgccccctattgacgtcaatgacggtaaatggcccgcctggcattatgcccagtacatgaccttatgggactttcctacttggcagtacatctacgtattagtcatcgctattaccatgctgatgcggttttggcagtacatcaatgggcgtggatagcggtttgactcacggggatttccaagtctccaccccattgacgtcaatgggagtttgttttggcaccaaaatcaacgggactttccaaaatgtcgtaacaactccgccccattgacgcaaatgggcggtaggcgtgtacggtgggaggtctatataagcagagct

SEQ ID NO: 12 - protein, 254 aa, synthetic construct
  REGION 1..254: note = laboratory made
MWQLLLPTALLLLVSAGMRTEDLPKAVVFLEPQWYRVLEKDSVTLKCQGAYSPEDNSTQWFHNESLISSQASSYFIDAATVDDSGEYRCQTNLSTLSDPVQLEVHIGWLLLQAPRWVFKEEDPIHLRCHSWKNTALHKVTYLQNGKGRKYFHHNSDFYIPKATLKDSGSYFCRGLVGSKNVSSETVNITITQGLAVSTISSFFPPGYQVSFCLVMVLLFAVDTGLYFSVKTNIRSSTRDWKDHKFKWRKDPQDK

SEQ ID NO: 13 - DNA, 765 bp, synthetic construct
  misc_feature 1..765: note = laboratory made
  source 1..765: mol_type = other DNA
atgtggcagctgctgctgcctacagctctcctgctgctggtgtccgccggcatgagaaccgaggatctgcctaaggccgtggtgttcctggaaccccagtggtacagagtgctggaaaaggacagcgtgaccctgaagtgccagggcgcctacagccccgaggacaatagcacccagtggttccacaacgagagcctgatcagcagccaggccagcagctacttcatcgacgccgccaccgtggacgacagcggcgagtatagatgccagaccaacctgagcaccctgagcgaccccgtgcagctggaagtgcacatcggatggctgctgctgcaggcccccagatgggtgttcaaagaagaggaccccatccacctgagatgccactcttggaagaacaccgccctgcacaaagtgacctacctgcagaacggcaagggcagaaagtacttccaccacaacagcgacttctacatccccaaggccaccctgaaggactccggctcctacttctgcagaggcctcgtgggcagcaagaacgtgtccagcgagacagtgaacatcaccatcacccagggcctggccgtgtctaccatcagcagctttttcccacccggctaccaggtgtccttctgcctcgtgatggtgctgctgttcgccgtggacaccggcctgtacttcagcgtgaaaacaaacatcagaagcagcacccgggactggaaggaccacaagttcaagtggcggaaggacccccaggacaagtga

SEQ ID NO: 14 - DNA, 483 bp, synthetic construct
  misc_feature 1..483: note = laboratory made
  source 1..483: mol_type = other DNA
atgtaccggatgcagctgctgagctgtatcgccctgtctctggccctcgtgaccaacagcgcccctaccagcagcagcaccaagaaaacccagctgcagctggaacatctgctgctggacctgcagatgatcctgaacggcatcaacaactacaagaaccccaagctgacccggatgctgaccttcaagttctacatgcccaagaaggccaccgaactgaaacatctgcagtgcctggaagaggaactgaagcccctggaagaagtgctgaacctggcccagagcaagaacttccacctgaggcccagggacctgatcagcaacatcaacgtgatcgtgctggaactgaaaggcagcgagacaaccttcatgtgcgagtacgccgacgagacagctaccatcgtggaatttctgaaccggtggatcaccttctgccagagcatcatcagcaccctgaccggctccgagaaggacgagctgtga

SEQ ID NO: 15 - protein, 164 aa, synthetic construct
  REGION 1..164: note = laboratory made
MYRMQLLSCIALSLALVTNSAPTSSSTKKTQLQLEHLLLDLQMILNGINNYKNPKLTRMLTFKFYMPKKATELKHLQCLEEELKPLEEVLNLAQSKNFHLRPRDLISNINVIVLELKGSETTFMCEYADETATIVEFLNRWITFCQSIISTLTGSEKDELKDEL

SEQ ID NO: 16 - DNA, 297 bp, synthetic construct
  misc_feature 1..297: note = laboratory made
  source 1..297: mol_type = other DNA
atggccctgctactggccctcagcctgctggttctctggacttccccagccccaactctgagtggcaccaatgatgctgaagactgctgcctgtctgtgacccagaaacccatccctgggtacatcgtgaggaacttccactaccttctcatcaaggatggctgcagggtgcctgctgtagtgttcaccacactgaggggccgccagctctgtgcacccccagaccagccctgggtagaacgcatcatccagagactgcagaggacctcagccaagatgaagcgccgcagcagttaa

SEQ ID NO: 17 - DNA, 60 bp, synthetic construct
  misc_feature 1..60: note = laboratory made
  source 1..60: mol_type = other DNA
cagtgcaccaactacgccctgctgaagctggccggcgacgtggagagcaaccctggccct

SEQ ID NO: 18 - DNA, 54 bp, synthetic construct
  misc_feature 1..54: note = laboratory made
  source 1..54: mol_type = other DNA
gagggcagaggcagcctgctgacctgcggcgatgtggaggaaaacccaggccca

SEQ ID NO: 19 - DNA, 806 bp, synthetic construct
  misc_feature 1..806: note = laboratory made
  source 1..806: mol_type = other DNA
tgctttctctgacctgcattctctcccctgggcctgtgccgctttctgtctgcagcttgtggcctgggtcacctctacggctggcccagatccttccctgccgcctccttcaggttccgtcttcctccactccctcttccccttgctctctgctgtgttgctgcccaaggatgctctttccggagcacttccttctcggcgctgcaccacgtgatgtcctctgagcggatcctccccgtgtctgggtcctctccgggcatctctcctccctcacccaaccccatgccgtcttcactcgctgggttcccttttccttctccttctggggcctgtgccatctctcgtttcttaggatggccttctccgacggatgtctcccttgcgtcccgcctccccttcttgtaggcctgcatcatcaccgtttttctggacaaccccaaagtaccccgtctccctggctttagccacctctccatcctcttgctttctttgcctggacaccccgttctcctgtggattcgggtcacctctcactcctttcatttgggcagctcccctaccccccttacctctctagtctgtgctagctcttccagccccctgtcatggcatcttccaggggtccgagagctcagctagtcttcttcctccaacccgggcccctatgtccacttcaggacagcatgtttgctgcctccagggatcctgtgtccccgagctgggaccaccttatattcccagggccggttaatgtggctctggttctgggtacttttatctgtcccctccaccccacagtggggtac

SEQ ID NO: 20 - DNA, 1178 bp, synthetic construct; identical to SEQ ID NO: 3
  misc_feature 1..1178: note = Laboratory made
  source 1..1178: mol_type = other DNA

SEQ ID NO: 21 - DNA, 19 bp, synthetic construct
  misc_feature 1..19: note = laboratory made
  source 1..19: mol_type = other DNA
taatacgactcactatagg

SEQ ID NO: 22 - DNA, 1116 bp, synthetic construct
  misc_feature 1..1116: note = laboratory made
  source 1..1116: mol_type = other DNA
atgaaaagcgtgctggtggtggctctccttgtcattttccaggtatgcctgtgtcaagatgaggtcacggacgattacatcggagacaacaccacagtggactacactttgttcgagtctttgtgctccaagaaggacgtgcggaactttaaagcctggttcctccctatcatgtactccatcatttgtttcgtgggcctactgggcaatgggctggtcgtgttgacctatatctatttcaagaggctcaagaccatgaccgatacctacctgctcaacctggcggtggcagacatcctcttcctcctgacccttcccttctgggcctacagcgcggccaagtcctgggtcttcggtgtccacttttgcaagctcatctttgccatctacaagatgagcttcttcagtggcatgctcctacttctttgcatcagcattgaccgctacgtggccatcgtccaggctgtctcagctcaccgccaccgtgcccgcgtccttctcatcagcaagctgtcctgtgtgggcatctggatactagccacagtgctctccatcccagagctcctgtacagtgacctccagaggagcagcagtgagcaagcgatgcgatgctctctcatcacagagcatgtggaggcctttatcaccatccaggtggcccagatggtgatcggctttctggtccccctgctggccatgagcttctgttaccttgtcatcatccgcaccctgctccaggcacgcaactttgagcgcaacaaggccatcaaggtgatcatcgctgtggtcgtggtcttcatagtcttccagctgccctacaatggggtggtcctggcccagacggtggccaacttcaacatcaccagtagcacctgtgagctcagtaagcaactcaacatcgcctacgacgtcacctacagcctggcctgcgtccgctgctgcgtcaaccctttcttgtacgccttcatcggcgtcaagttccgcaacgatctcttcaagctcttcaaggacctgggctgcctcagccaggagcagctccggcagtggtcttcctgtcggcacatccggcgctcctccatgagtgtggaggccgagaccaccaccaccttctcccca

SEQ ID NO: 23 - DNA, 66 bp, synthetic construct
  misc_feature 1..66: note = laboratory made
  source 1..66: mol_type = other DNA
ggatctggagctactaacttcagcctgctgaagcaggctggagacgtggaggagaaccctggacct

SEQ ID NO: 24 - DNA, 69 bp, synthetic construct
  misc_feature 1..69: note = laboratory made
  source 1..69: mol_type = other DNA
atggactggatctggcggattctgtttctcgtgggagctgccacaggcgctcattctgctcagcctgcc

SEQ ID NO: 25 - DNA, 1152 bp, synthetic construct
  misc_feature 1..1152: note = laboratory made
  source 1..1152: mol_type = other DNA
gatatccagatgacccagacaacaagcagcctgagcgcctctctgggcgatagagtgacaatcagctgcagagccagccaggacatcagcaagtacctgaactggtatcagcagaaacccgacggcaccgtgaagctgctgatctaccacacaagcagactgcacagcggcgtgccaagcagattttctggcagcggcagcggcaccgattacagcctgaccatcagcaacctggaacaggaagatatcgctacctacttctgtcagcagggcaacaccctgccttacacctttggcggcggaacaaagctggaactgaaaagaggcggcggaggaagcggaggcggaggatctgggggcggaggctctggcggagggggatctgaagtgcagctgcagcagtctggacctggactggtggctccttctcagtccctgtctgtgacctgtacagtgtctggcgtgtccctgcctgattacggcgtgtcctggatcagacagcctcccagaaaaggcctggaatggctgggagtgatctggggcagcgagacaacctactacaacagcgccctgaagtcccggctgaccatcatcaaggacaacagcaagagccaggtgttcctgaagatgaacagcctgcagaccgacgacaccgccatctactactgcgccaagcactactactacggcggcagctacgccatggattattggggccagggcaccaccgtgacagtgtcatctgcggccgcgctgagcaacagcatcatgtacttcagccacttcgtgcctgtgttcctgcctgccaagcctacaacaacaccagcccctagacctccaacccctgcccctacaattgcctctcagcctctgtctctgaggcccgaagcttgtagacctgctgctggcggagctgtgcacaccagaggactggatttcgcctgcttttgggtgctggtggtcgtgggcggagtgctggcttgttattctctgctggtcaccgtggccttcatcatcttttgggtccgactgaagatccaggtccgaaaggccgccatcaccagctacgagaagtctgatggcgtgtacaccggcctgagcaccagaaaccaggaaacctacgagacactgaagcacgagaagcccccccag

SEQ ID NO: 26 - DNA, 765 bp, synthetic construct; identical to SEQ ID NO: 13
  misc_feature 1..765: note = laboratory made
  source 1..765: mol_type = other DNA

SEQ ID NO: 27 - DNA, 597 bp, synthetic construct
  misc_feature 1..597: note = laboratory made
  source 1..597: mol_type = other DNA
aattccgcccctctcccccccccccctctccctcccccccccctaacgttactggccgaagccgcttggaataaggccggtgtgcgtttgtctatatgttattttccaccatattgccgtcttttggcaatgtgagggcccggaaacctggccctgtcttcttgacgagcattcctaggggtctttcccctctcgccaaaggaatgcaaggtctgttgaatgtcgtgaaggaagcagttcctctggaagcttcttgaagacaaacaacgtctgtagcgaccctttgcaggcagcggaaccccccacctggcgacaggtgcctctgcggccaaaagccacgtgtataagatacacctgcaaaggcggcacaaccccagtgccacgttgtgagttggatagttgtggaaagagtcaaatggctctcctcaagcgtattcaacaaggggctgaaggatgcccagaaggtaccccattgtatgggatctgatctggggcctcggtgcacatgctttacatgtgtttagtcgaggttaaaaaaacgtctaggccccccgaaccacggggacgtggttttcctttgaaaaacacgataaccgc

SEQ ID NO: 28 - DNA, 483 bp, synthetic construct; identical to SEQ ID NO: 14
  misc_feature 1..483: note = laboratory made
  source 1..483: mol_type = other DNA

SEQ ID NO: 29 - DNA, 252 bp, synthetic construct
  misc_feature 1..252: note = laboratory made
  source 1..252: mol_type = other DNA
acgagatttcgattccaccgccgccttctatgaaaggttgggcttcggaatcgttttccgggacgccggctggatgatcctccagcgcggggatctcatgctggagttcttcgcccaccccaacttgtttattgcagcttataatggttacaaataaagcaatagcatcacaaatttcacaaataaagcatttttttcactgcattctagttgtggtttgtccaaactcatcaatgtatcttatcatgtctg

SEQ ID NO: 30 - DNA, 844 bp, synthetic construct
  misc_feature 1..844: note = laboratory made
  source 1..844: mol_type = other DNA
ctagggacaggattggtgacagaaaagccccatccttaggcctcctccttcctagtctcctgatattgggtctaacccccacctcctgttaggcagattccttatctggtgacacacccccatttcctggagccatctctctccttgccagaacctctaaggtttgcttacgatggagccagagaggatcctgggagggagagcttggcagggggtgggagggaagggggggatgcgtgacctgcccggttctcagtggccaccctgcgctaccctctcccagaacctgagctgctctgacgcggctgtctggtgcgtttcactgatcctggtgctgcagcttccttacacttcccaagaggagaagcagtttggaaaaacaaaatcagaataagttggtcctgagttctaactttggctcttcacctttctagtccccaatttatattgttcctccgtgcgtcagttttacctgtgagataaggccagtagccagccccgtcctggcagggctgtggtgaggaggggggtgtccgtgtggaaaactccctttgtgagaatggtgcgtcctaggtgttcaccaggtcgtggccgcctctactccctttctctttctccatccttctttccttaaagagtccccagtgctatctgggacatattcctccgcccagagcagggtcccgcttccctaaggccctgctctgggcttctgggtttgagtccttggcaagcccaggagaggcgctcaggcttccctgtcccccttcctcgtccaccatctcatgcccctggctctcctgccccttccctacaggggttcctggctctgctcttcagactg

SEQ ID NO: 31 - protein, 41 aa, synthetic construct
  REGION 1..41: note = laboratory made
LKIQVRKAAITSYEKSDGVYTGLSTRNQETYETLKHEKPPQ

SEQ ID NO: 32 - DNA, 123 bp, synthetic construct
  misc_feature 1..123: note = laboratory made
  source 1..123: mol_type = other DNA
ctgaagatccaggtccgaaaggccgccatcaccagctacgagaagtctgatggcgtgtacaccggcctgagcaccagaaaccaggaaacctacgagacactgaagcacgagaagcccccccag

SEQ ID NO: 33 - protein, 64 aa, synthetic construct
  REGION 1..64: note = laboratory made
LSNSIMYFSHFVPVFLPAKPTTTPAPRPPTPAPTIASQPLSLRPEACRPAAGGAVHTRGLDFAC

SEQ ID NO: 34 - DNA, 192 bp, synthetic construct
  misc_feature 1..192: note = laboratory made
  source 1..192: mol_type = other DNA
ctgagcaacagcatcatgtacttcagccacttcgtgcctgtgttcctgcctgccaagcctacaacaacaccagcccctagacctccaacccctgcccctacaattgcctctcagcctctgtctctgaggcccgaagcttgtagacctgctgctggcggagctgtgcacaccagaggactggatttcgcctgc

SEQ ID NO: 35 - protein, 28 aa, synthetic construct
  REGION 1..28: note = laboratory made
FWVLVVVGGVLACYSLLVTVAFIIFWVR

SEQ ID NO: 36 - DNA, 84 bp, synthetic construct
  misc_feature 1..84: note = laboratory made
  source 1..84: mol_type = other DNA
ttttgggtgctggtggtcgtgggcggagtgctggcttgttattctctgctggtcaccgtggccttcatcatcttttgggtccga

SEQ ID NO: 37 - protein, 133 aa, synthetic construct
  REGION 1..133: note = laboratory made
LSNSIMYFSHFVPVFLPAKPTTTPAPRPPTPAPTIASQPLSLRPEACRPAAGGAVHTRGLDFACFWVLVVVGGVLACYSLLVTVAFIIFWVRLKIQVRKAAITSYEKSDGVYTGLSTRNQETYETLKHEKPPQ

SEQ ID NO: 38 - DNA, 399 bp, synthetic construct
  misc_feature 1..399: note = laboratory made
  source 1..399: mol_type = other DNA
ctgagcaacagcatcatgtacttcagccacttcgtgcctgtgttcctgcctgccaagcctacaacaacaccagcccctagacctccaacccctgcccctacaattgcctctcagcctctgtctctgaggcccgaagcttgtagacctgctgctggcggagctgtgcacaccagaggactggatttcgcctgcttttgggtgctggtggtcgtgggcggagtgctggcttgttattctctgctggtcaccgtggccttcatcatcttttgggtccgactgaagatccaggtccgaaaggccgccatcaccagctacgagaagtctgatggcgtgtacaccggcctgagcaccagaaaccaggaaacctacgagacactgaagcacgagaagcccccccag

SEQ ID NO: 39 - protein, 252 aa, synthetic construct
  REGION 1..252: note = laboratory made
AQPADIQMTQTTSSLSASLGDRVTISCRASQDISKYLNWYQQKPDGTVKLLIYHTSRLHSGVPSRFSGSGSGTDYSLTISNLEQEDIATYFCQQGNTLPYTFGGGTKLELKRGGGGSGGGGSGGGGSGGGGSEVQLQQSGPGLVAPSQSLSVTCTVSGVSLPDYGVSWIRQPPRKGLEWLGVIWGSETTYYNSALKSRLTIIKDNSKSQVFLKMNSLQTDDTAIYYCAKHYYYGGSYAMDYWGQGTTVTVSS

SEQ ID NO: 40 - protein, 113 aa, synthetic construct
  REGION 1..113: note = laboratory made
RVKFSRSADAPAYQQGQNQLYNELNLGRREEYDVLDKRRGRDPEMGGKPQRRKNPQEGLYNELQKDKMAEAYSEIGMKGERRRGKGHDGLYQGLSTATKDTYDALHMQALPPR

SEQ ID NO: 41 - DNA, 1410 bp, synthetic construct
  misc_feature 1..1410: note = laboratory made
  source 1..1410: mol_type = other DNA
atggactggatctggcggatcctgtttctcgtgggagctgccacaggcgctcattctgctcagcctgccgatatccagatgacccagacaacaagcagcctgagcgcctctctgggcgatagagtgacaatcagctgcagagccagccaggacatcagcaagtacctgaactggtatcagcagaaacccgacggcaccgtgaagctgctgatctaccacacaagcagactgcacagcggcgtgccaagcagattttctggcagcggcagcggcaccgattacagcctgaccatcagcaacctggaacaggaagatatcgctacctacttctgtcagcaaggcaacaccctgccttacacctttggcggcggaacaaagctggaactgaaaagaggcggcggaggaagcggaggcggaggatctgggggcggaggctctggcggagggggatctgaagtgcagctgcagcagtctggacctggactggtggctccttctcagtccctgtctgtgacctgtacagtgtctggcgtgtccctgcctgattacggcgtgtcctggatcagacagcctcccagaaaaggcctggaatggctgggagtgatctggggcagcgagacaacctactacaacagcgccctgaagtcccggctgaccatcatcaaggacaacagcaagagccaggtgttcctgaagatgaacagcctgcagaccgacgacaccgccatctactactgcgccaagcactactactacggcggcagctacgccatggattattggggccagggcaccaccgtgacagtgtcatctgctgctgctctgttcgtgcctgtgttcctgcctgccaagcctacaacaacaccagcccctagacctccaacccctgcccctacaattgcctctcagcctctgtctctgaggcccgaagcttgtagacctgctgctggcggagctgtgcacaccagaggactggatttcgcctgcttttgggtgctggtggtcgtgggcggagtgctggcttgttattctctgctggtcaccgtggccttcatcatcttttgggtccgagtgaagttcagcagatccgccgatgcccctgcttaccagcagggccagaatcagctgtacaacgagctgaacctgggcagacgggaagagtacgacgtgctggataagagaagaggcagagatcccgagatgggcggcaagccccagagaagaaagaatccccaggaaggcctgtataacgaactgcagaaagacaagatggccgaggcctacagcgagatcggcatgaagggcgagagaagaagaggcaagggccacgatggactgtaccagggactgagcacagccaccaaggatacctacgatgccctgcacatgcaggccctgcctccaagataa

SEQ ID NO: 42 - protein, 153 aa, synthetic construct
  REGION 1..153: note = laboratory made
MYRMQLLSCIALSLALVTNSAPTSSSTKKTQLQLEHLLLDLQMILNGINNYKNPKLTRMLTFKFYMPKKATELKHLQCLEEELKPLEEVLNLAQSKNFHLRPRDLISNINVIVLELKGSETTFMCEYADETATIVEFLNRWITFCQSIISTLT

SEQ ID NO: 43 - protein, 160 aa, synthetic construct
  REGION 1..160: note = laboratory made
MYRMQLLSCIALSLALVTNSAPTSSSTKKTQLQLEHLLLDLQMILNGINNYKNPKLTRMLTFKFYMPKKATELKHLQCLEEELKPLEEVLNLAQSKNFHLRPRDLISNINVIVLELKGSETTFMCEYADETATIVEFLNRWITFCQSIISTLTGSEKDEL

SEQ ID NO: 44 - protein, 372 aa, synthetic construct
  REGION 1..372: note = laboratory made
MKSVLVVALLVIFQVCLCQDEVTDDYIGDNTTVDYTLFESLCSKKDVRNFKAWFLPIMYSIICFVGLLGNGLVVLTYIYFKRLKTMTDTYLLNLAVADILFLLTLPFWAYSAAKSWVFGVHFCKLIFAIYKMSFFSGMLLLLCISIDRYVAIVQAVSAHRHRARVLLISKLSCVGIWILATVLSIPELLYSDLQRSSSEQAMRCSLITEHVEAFITIQVAQMVIGFLVPLLAMSFCYLVIIRTLLQARNFERNKAIKVIIAVVVVFIVFQLPYNGVVLAQTVANFNITSSTCELSKQLNIAYDVTYSLACVRCCVNPFLYAFIGVKFRNDLFKLFKDLGCLSQEQLRQWSSCRHIRRSSMSVEAETTTTFSP

SEQ ID NO: 45 - protein, 98 aa, synthetic construct
  REGION 1..98: note = laboratory made
MALLLALSLLVLWTSPAPTLSGTNDAEDCCLSVTQKPIPGYIVRNFHYLLIKDGCRVPAVVFTTLRGRQLCAPPDQPWVERIIQRLQRTSAKMKRRSS

SEQ ID NO: 46 - protein, 134 aa, synthetic construct
  REGION 1..134: note = laboratory made
MAQSLALSLLILVLAFGIPRTQGSDGGAQDCCLKYSQRKIPAKVVRSYRKQEPSLGCSIPAILFLPRKRSQAELCADPKELWVQQLMQHLDKTPSPQKPAQGCRKDRGASKTGKKGKGSKGCKRTERSQTPKGP

SEQ ID NO: 47 - DNA, 1083 bp, synthetic construct
  misc_feature 1..1083: note = laboratory made
  source 1..1083: mol_type = other DNA
atggaagattttaacatggagagtgacagctttgaagatttctggaaaggtgaagatcttagtaattacagttacagctctaccctgcccccttttctactagatgccgccccatgtgaaccagaatccctggaaatcaacaagtattttgtggtcattatctatgccctggtattcctgctgagcctgctgggaaactccctcgtgatgctggtcatcttatacagcagggtcggccgctccgtcactgatgtctacctgctgaacctagccttggccgacctactctttgccctgaccttgcccatctgggccgcctccaaggtgaatggctggatttttggcacattcctgtgcaaggtggtctcactcctgaaggaagtcaacttctatagtggcatcctgctactggcctgcatcagtgtggaccgttacctggccattgtccatgccacacgcacactgacccagaagcgctacttggtcaaattcatatgtctcagcatctggggtctgtccttgctcctggccctgcctgtcttacttttccgaaggaccgtctactcatccaatgttagcccagcctgctatgaggacatgggcaacaatacagcaaactggcggatgctgttacggatcctgccccagtcctttggcttcatcgtgccactgctgatcatgctgttctgctacggattcaccctgcgtacgctgtttaaggcccacatggggcagaagcaccgggccatgcgggtcatctttgctgtcgtcctcatcttcctgctctgctggctgccctacaacctggtcctgctggcagacaccctcatgaggacccaggtgatccaggagacctgtgagcgccgcaatcacatcgaccgggctctggatgccaccgagattctgggcatccttcacagctgcctcaaccccctcatctacgccttcattggccagaagtttcgccatggactcctcaagattctagctatacatggcttgatcagcaaggactccctgcccaaagacagcaggccttcctttgttggctcttcttcagggcacacttccactactctctaa

SEQ ID NO: 48 - protein, 360 aa, synthetic construct
  REGION 1..360: note = laboratory made
MEDFNMESDSFEDFWKGEDLSNYSYSSTLPPFLLDAAPCEPESLEINKYFVVIIYALVFLLSLLGNSLVMLVILYSRVGRSVTDVYLLNLALADLLFALTLPIWAASKVNGWIFGTFLCKVVSLLKEVNFYSGILLLACISVDRYLAIVHATRTLTQKRYLVKFICLSIWGLSLLLALPVLLFRRTVYSSNVSPACYEDMGNNTANWRMLLRILPQSFGFIVPLLIMLFCYGFTLRTLFKAHMGQKHRAMRVIFAVVLIFLLCWLPYNLVLLADTLMRTQVIQETCERRNHIDRALDATEILGILHSCLNPLIYAFIGQKFRHGLLKILAIHGLISKDSLPKDSRPSFVGSSSGHTSTTL

SEQ ID NO: 49 - DNA, 336 bp, synthetic construct
  misc_feature 1..336: note = laboratory made
  source 1..336: mol_type = other DNA
atgtccctgctcccacgccgcgcccctccggtcagcatgaggctcctggcggccgcgctgctcctgctgctgctggcgctgtacaccgcgcgtgtggacgggtccaaatgcaagtgctcccggaagggacccaagatccgctacagcgacgtgaagaagctggaaatgaagccaaagtacccgcactgcgaggagaagatggttatcatcaccaccaagagcgtgtccaggtaccgaggtcaggagcactgcctgcaccccaagctgcagagcaccaagcgcttcatcaagtggtacaacgcctggaacgagaagcgcagggtctacgaagaatag

SEQ ID NO: 50 - protein, 111 aa, synthetic construct
  REGION 1..111: note = laboratory made
MSLLPRRAPPVSMRLLAAALLLLLLALYTARVDGSKCKCSRKGPKIRYSDVKKLEMKPKYPHCEEKMVIITTKSVSRYRGQEHCLHPKLQSTKRFIKWYNAWNEKRRVYEE

SEQ ID NO: 51 - DNA, 1119 bp, synthetic construct
  misc_feature 1..1119: note = laboratory made
  source 1..1119: mol_type = other DNA
atgatatttccatggaaatgtcagagcacccagagggacttatggaacatcttcaagttgtgggggtggacaatgctctgttgtgatttcctggcacatcatggaaccgactgctggacttaccattattctgaaaaacccatgaactggcaaagggctagaagattctgccgagacaattacacagatttagttgccatacaaaacaaggcggaaattgagtatctggagaagactctgcctttcagtcgttcttactactggataggaatccggaagataggaggaatatggacgtgggtgggaaccaacaaatctcttactgaagaagcagagaactggggagatggtgagcccaacaacaagaagaacaaggaggactgcgtggagatctatatcaagagaaacaaagatgcaggcaaatggaacgatgacgcctgccacaaactaaaggcagccctctgttacacagcttcttgccagccctggtcatgcagtggccatggagaatgtgtagaaatcatcaataattacacctgcaactgtgatgtggggtactatgggccccagtgtcagtttgtgattcagtgtgagcctttggaggccccagagctgggtaccatggactgtactcaccctttgggaaacttcagcttcagctcacagtgtgccttcagctgctctgaaggaacaaacttaactgggattgaagaaaccacctgtggaccatttggaaactggtcatctccagaaccaacctgtcaagtgattcagtgtgagcctctatcagcaccagatttggggatcatgaactgtagccatcccctggccagcttcagctttacctctgcatgtaccttcatctgctcagaaggaactgagttaattgggaagaagaaaaccatttgtgaatcatctggaatctggtcaaatcctagtccaatatgtcaaaaattggacaaaagtttctcaatgattaaggagggtgattataaccccctcttcattccagtggcagtcatggttactgcattctctgggttggcatttatcatttggctggcaaggagattaaaaaaaggcaagaaatccaagagaagtatgaatgacccatattaa

SEQ ID NO: 52 - protein, 372 aa, synthetic construct [sequence omitted]

SEQ ID NO: 53 - DNA, 300 bp, synthetic construct
  misc_feature 1..300: note = laboratory made
  source 1..300: mol_type = other DNA
atgacttccaagctggccgtggctctcttggcagccttcctgatttctgcagctctgtgtgaaggtgcagttttgccaaggagtgctaaagaacttagatgtcagtgcataaagacatactccaaacctttccaccccaaatttatcaaagaactgagagtgattgagagtggaccacactgcgccaacacagaaattattgtaaagctttctgatggaagagagctctgtctggaccccaaggaaaactgggtgcagagggttgtggagaagtttttgaagagggctgagaattcataa

SEQ ID NO: 54 - protein, 99 aa, synthetic construct
  REGION 1..99: note = laboratory made
MTSKLAVALLAAFLISAALCEGAVLPRSAKELRCQCIKTYSKPFHPKFIKELRVIESGPHCANTEIIVKLSDGRELCLDPKENWVQRVVEKFLKRAENS

SEQ ID NO: 55 - DNA, 324 bp, synthetic construct
  misc_feature 1..324: note = laboratory made
  source 1..324: mol_type = other DNA
atggcccgcgctgctctctccgccgcccccagcaatccccggctcctgcgagtggcactgctgctcctgctcctggtagccgctggccggcgcgcagcaggagcgtccgtggccactgaactgcgctgccagtgcttgcagaccctgcagggaattcaccccaagaacatccaaagtgtgaacgtgaagtcccccggaccccactgcgcccaaaccgaagtcatagccacactcaagaatgggcggaaagcttgcctcaatcctgcatcccccatagttaagaaaatcatcgaaaagatgctgaacagtgacaaatccaactga

SEQ ID NO: 56 - protein, 107 aa, synthetic construct
  REGION 1..107: note = laboratory made
MARAALSAAPSNPRLLRVALLLLLLVAAGRRAAGASVATELRCQCLQTLQGIHPKNIQSVNVKSPGPHCAQTEVIATLKNGRKACLNPASPIVKKIIEKMLNSDKSN

SEQ ID NO: 57 - DNA, 762 bp, synthetic construct
  misc_feature 1..762: note = laboratory made
  source 1..762: mol_type = other DNA
atgtggccccctgggtcagcctcccagccaccgccctcacctgccgcggccacaggtctgcatccagcggctcgccctgtgtccctgcagtgccggctcagcatgtgtccagcgcgcagcctcctccttgtggctaccctggtcctcctggaccacctcagtttggccagaaacctccccgtggccactccagacccaggaatgttcccatgccttcaccactcccaaaacctgctgagggccgtcagcaacatgctccagaaggccagacaaactctagaattttacccttgcacttctgaagagattgatcatgaagatatcacaaaagataaaaccagcacagtggaggcctgtttaccattggaattaaccaagaatgagagttgcctaaattccagagagacctctttcataactaatgggagttgcctggcctccagaaagacctcttttatgatggccctgtgccttagtagtatttatgaagacttgaagatgtaccaggtggagttcaagaccatgaatgcaaagcttctgatggatcctaagaggcagatctttctagatcaaaacatgctggcagttattgatgagctgatgcaggccctgaatttcaacagtgagactgtgccacaaaaatcctcccttgaagaaccggatttttataaaactaaaatcaagctctgcatacttcttcatgctttcagaattcgggcagtgactattgatagagtgatgagctatctgaatgcttcctaa

SEQ ID NO: 58 - protein, 253 aa, synthetic construct
  REGION 1..253: note = laboratory made
MWPPGSASQPPPSPAAATGLHPAARPVSLQCRLSMCPARSLLLVATLVLLDHLSLARNLPVATPDPGMFPCLHHSQNLLRAVSNMLQKARQTLEFYPCTSEEIDHEDITKDKTSTVEACLPLELTKNESCLNSRETSFITNGSCLASRKTSFMMALCLSSIYEDLKMYQVEFKTMNAKLLMDPKRQIFLDQNMLAVIDELMQALNFNSETVPQKSSLEEPDFYKTKIKLCILLHAFRIRAVTIDRVMSYLNAS

SEQ ID NO: 59 - DNA, 987 bp, synthetic construct
  misc_feature 1..987: note = laboratory made
  source 1..987: mol_type = other DNA
atgtgtcaccagcagttggtcatctcttggttttccctggtttttctggcatctcccctcgtggccatatgggaactgaagaaagatgtttatgtcgtagaattggattggtatccggatgcccctggagaaatggtggtcctcacctgtgacacccctgaagaagatggtatcacctggaccttggaccagagcagtgaggtcttaggctctggcaaaaccctgaccatccaagtcaaagagtttggagatgctggccagtacacctgtcacaaaggaggcgaggttctaagccattcgctcctgctgcttcacaaaaaggaagatggaatttggtccactgatattttaaaggaccagaaagaacccaaaaataagacctttctaagatgcgaggccaagaattattctggacgtttcacctgctggtggctgacgacaatcagtactgatttgacattcagtgtcaaaagcagcagaggctcttctgacccccaaggggtgacgtgcggagctgctacactctctgcagagagagtcagaggggacaacaaggagtatgagtactcagtggagtgccaggaggacagtgcctgcccagctgctgaggagagtctgcccattgaggtcatggtggatgccgttcacaagctcaagtatgaaaactacaccagcagcttcttcatcagggacatcatcaaacctgacccacccaagaacttgcagctgaagccattaaagaattctcggcaggtggaggtcagctgggagtaccctgacacctggagtactccacattcctacttctccctgacattctgcgttcaggtccagggcaagagcaagagagaaaagaaagatagagtcttcacggacaagacctcagccacggtcatctgccgcaaaaatgccagcattagcgtgcgggcccaggaccgctactatagctcatcttggagcgaatgggcatctgtgccctgcagttag

SEQ ID NO: 60 - protein, 328 aa, synthetic construct
  REGION 1..328: note = laboratory made
MCHQQLVISWFSLVFLASPLVAIWELKKDVYVVELDWYPDAPGEMVVLTCDTPEEDGITWTLDQSSEVLGSGKTLTIQVKEFGDAGQYTCHKGGEVLSHSLLLLHKKEDGIWSTDILKDQKEPKNKTFLRCEAKNYSGRFTCWWLTTISTDLTFSVKSSRGSSDPQGVTCGAATLSAERVRGDNKEYEYSVECQEDSACPAAEESLPIEVMVDAVHKLKYENYTSSFFIRDIIKPDPPKNLQLKPLKNSRQVEVSWEYPDTWSTPHSYFSLTFCVQVQGKSKREKKDRVFTDKTSATVICRKNASISVRAQDRYYSSSWSEWASVPCS

SEQ ID NO: 61 - protein, 536 aa, synthetic construct
  REGION 1..536: note = laboratory made
MGHQQLVISWFSLVFLASPLVAIWELKKDVYVVELDWYPDAPGEMVVLTCDTPEEDGITWTLDQSSEVLGSGKTLTIQVKEFGDAGQYTCHKGGEVLSHSLLLLHKKEDGIWSTDILKDQKEPKNKTFLRCEAKNYSGRFTCWWLTTISTDLTFSVKSSRGSSDPQGVTCGAATLSAERVRGDNKEYEYSVECQEDSACPAAEESLPIEVMVDAVHKLKYENYTSSFFIRDIIKPDPPKNLQLKPLKNSRQVEVSWEYPDTWSTPHSYFSLTFCVQVQGKSKREKKDRVFTDKTSATVICRKNASISVRAQDRYYSSSWSEWASVPCSVPGVGVPGVGARNLPVATPDPGMFPCLHHSQNLLRAVSNMLQKARQTLEFYPCTSEEIDHEDITKDKTSTVEACLPLELTKNESCLNSRETSFITNGSCLASRKTSFMMALCLSSIYEDSKMYQVEFKTMNAKLLMDPKRQIFLDQNMLAVIDELMQALNFNSETVPQKSSLEEPDFYKTKIKLCILLHAFRIRAVTIDRVMSYLNAS

SEQ ID NO: 62 - DNA, 1611 bp, synthetic construct
  misc_feature 1..1611: note = laboratory made
  source 1..1611: mol_type = other DNA
atgggtcaccagcagttggtcatctcttggttttccctggtttttctggcatctcccctcgtggccatatgggaactgaagaaagatgtttatgtcgtagaattggattggtatccggatgcccctggagaaatggtggtcctcacctgtgacacccctgaagaagatggtatcacctggaccttggaccagagcagtgaggtcttaggctctggcaaaaccctgaccatccaagtcaaagagtttggagatgctggccagtacacctgtcacaaaggaggcgaggttctaagccattcgctcctgctgcttcacaaaaaggaagatggaatttggtccactgatattttaaaggaccagaaagaacccaaaaataagacctttctaagatgcgaggccaagaattattctggacgtttcacctgctggtggctgacgacaatcagtactgatttgacattcagtgtcaaaagcagcagaggctcttctgacccccaaggggtgacgtgcggagctgctacactctctgcagagagagtcagaggggacaacaaggagtatgagtactcagtggagtgccaggaggacagtgcctgcccagctgctgaggagagtctgcccattgaggtcatggtggatgccgttcacaagctcaagtatgaaaactacaccagcagcttcttcatcagggacatcatcaaacctgacccacccaagaacttgcagctgaagccattaaagaattctcggcaggtggaggtcagctgggagtaccctgacacctggagtactccacattcctacttctccctgacattctgcgttcaggtccagggcaagagcaagagagaaaagaaagatagagtcttcacggacaagacctcagccacggtcatctgccgcaaaaatgccagcattagcgtgcgggcccaggaccgctactatagctcatcttggagcgaatgggcatctgtgccctgcagtgttcctggagtaggggtacctggggtgggcgccagaaacctccccgtggccactccagacccaggaatgttcccatgccttcaccactcccaaaacctgctgagggccgtcagcaacatgctccagaaggccagacaaactctagaattttacccttgcacttctgaagagattgatcatgaagatatcacaaaagataaaaccagcacagtggaggcctgtttaccattggaattaaccaagaatgagagttgcctaaattccagagagacctctttcataactaatgggagttgcctggcctccagaaagacctcttttatgatggccctgtgccttagtagtatttatgaagactcgaagatgtaccaggtggagttcaagaccatgaatgcaaagcttctgatggatcctaagaggcagatctttctagatcaaaacatgctggcagttattgatgagctgatgcaggccctgaatttcaacagtgagactgtgccacaaaaatcctcccttgaagaaccggatttttataaaactaaaatcaagctctgcatacttcttcatgctttcagaattcgggcagtgactattgatagagtgatgagctatctgaatgcttcctaa

SEQ ID NO: 63 - DNA, 477 bp, synthetic construct
  misc_feature 1..477: note = laboratory made
  source 1..477: mol_type = other DNA
atgggtcgggggctgctcaggggcctgtggccgctgcacatcgtcctgtggacgcgtatcgccagcacgatcccaccgcacgttcagaagtcggttaataacgacatgatagtcactgacaacaacggtgcagtcaagtttccacaactgtgtaaattttgtgatgtgagattttccacctgtgacaaccagaaatcctgcatgagcaactgcagcatcacctccatctgtgagaagccacaggaagtctgtgtggctgtatggagaaagaatgacgagaacataacactagagacagtttgccatgaccccaagctcccctaccatgactttattctggaagatgctgcttctccaaagtgcattatgaaggaaaaaaaaaagcctggtgagactttcttcatgtgttcctgtagctctgatgagtgcaatgacaacatcatcttctcagaagaatataacaccagcaatcctgac

SEQ ID NO: 64 - protein, 159 aa, synthetic construct
  REGION 1..159: note = laboratory made
MGRGLLRGLWPLHIVLWTRIASTIPPHVQKSVNNDMIVTDNNGAVKFPQLCKFCDVRFSTCDNQKSCMSNCSITSICEKPQEVCVAVWRKNDENITLETVCHDPKLPYHDFILEDAASPKCIMKEKKKPGETFFMCSCSSDECNDNIIFSEEYNTSNPD

SEQ ID NO: 65 - DNA, 933 bp, synthetic construct
  misc_feature 1..933: note = laboratory made
  source 1..933: mol_type = other DNA
atgggtcgggggctgctcaggggcctgtggccgctgcacatcgtcctgtggacgcgtatcgccagcacgatcccaccgcacgttcagaagtcggttaataacgacatgatagtcactgacaacaacggtgcagtcaagtttccacaactgtgtaaattttgtgatgtgagattttccacctgtgacaaccagaaatcctgcatgagcaactgcagcatcacctccatctgtgagaagccacaggaagtctgtgtggctgtatggagaaagaatgacgagaacataacactagagacagtttgccatgaccccaagctcccctaccatgactttattctggaagatgctgcttctccaaagtgcattatgaaggaaaaaaaaaagcctggtgagactttcttcatgtgttcctgtagctctgatgagtgcaatgacaacatcatcttctcagaagaatataacaccagcaatcctgacggaggtggaggaagtggaggaggtggaagtggtggtggaggtagtacgatcccaccgcacgttcagaagtcggttaataacgacatgatagtcactgacaacaacggtgcagtcaagtttccacaactgtgtaaattttgtgatgtgagattttccacctgtgacaaccagaaatcctgcatgagcaactgcagcatcacctccatctgtgagaagccacaggaagtctgtgtggctgtatggagaaagaatgacgagaacataacactagagacagtttgccatgaccccaagctcccctaccatgactttattctggaagatgctgcttctccaaagtgcattatgaaggaaaaaaaaaagcctggtgagactttcttcatgtgttcctgtagctctgatgagtgcaatgacaacatcatcttctcagaagaatataacaccagcaatcctgac

SEQ ID NO: 66 - protein, 311 aa, synthetic construct
  REGION 1..311: note = laboratory made
MGRGLLRGLWPLHIVLWTRIASTIPPHVQKSVNNDMIVTDNNGAVKFPQLCKFCDVRFSTCDNQKSCMSNCSITSICEKPQEVCVAVWRKNDENITLETVCHDPKLPYHDFILEDAASPKCIMKEKKKPGETFFMCSCSSDECNDNIIFSEEYNTSNPDGGGGSGGGGSGGGGSTIPPHVQKSVNNDMIVTDNNGAVKFPQLCKFCDVRFSTCDNQKSCMSNCSITSICEKPQEVCVAVWRKNDENITLETVCHDPKLPYHDFILEDAASPKCIMKEKKKPGETFFMCSCSSDECNDNIIFSEEYNTSNPD

SEQ ID NO: 67 - DNA, 510 bp, synthetic construct
  misc_feature 1..510: note = Laboratory made
  source 1..510: mol_type = other DNA
atgcgcatcagcaagccccacctgcgcagcatcagcatccagtgctacctgtgcctgctgctgaacagccacttcctgaccgaggccggcatccacgtgttcatcctgggctgcttcagcgccggcctgcccaagaccgaggccaactgggtgaacgtgatcagcgacctgaagaagatcgaggacctgatccagagcatgcacatcgacgccaccctgtacaccgagagcgacgtgcaccccagctgcaaggtgaccgccatgaagtgcttcctgctggagctgcaggtgatcagcctggagagcggcgacgccagcatccacgacaccgtggagaacctgatcatcctggccaacaacagcctgagcagcaacggcaacgtgaccgagagcggctgcaaggagtgcgaggagctggaggagaagaacatcaaggagttcctgcagagcttcgtgcacatcgtgcagatgttcatcaacaccagcggctccgagaaggacgagctgtaa

SEQ ID NO: 68 - DNA, 1215 bp, synthetic construct
  misc_feature 1..1215: note = Laboratory made
  source 1..1215: mol_type = other DNA
atggactggatctggcggattctgtttctcgtgggagctgccacaggcgctcattctgctcagcctgccaacatccagatgacccagtctccatcttctgtgtctgcatctgtaggagacagagtcaccatcacttgtcgggcgagtcaggatattagccgctggttagcctggtatcagcagaaaccagggaaagcccctaaactcctgatctatgctgcatccagtttgcaaagtggggtcccatcgaggttcagcggcagtggatctgggacagatttcgctctcactatcagcagcctgcagcctgaagattttgcaacttactattgtcaacaggctgacagtcgtttctcgatcaccttcggccaagggacacgactggagattaaaggcggcggaggaagcggaggcggaggatctgggggcggaggctctggcggagggggatctgaggtgcagctggtgcagtctgggggaggcttggtacagcctggggggtccctgagactctcctgtgcagcctctggattcaccttcagtagctatagcatgaactgggtccgccaggctccagggaaggggctggagtgggtttcatacattagtagtagtagtagtaccatacagtacgcagactctgtgaagggccgattcaccatctccagagacaatgccaagaactcactgtatctgcaaatgaacagcctgagagacgaggacacggctgtgtattactgtgcgagaggggactactactacggtatggacgtctggggccaagggaccacggtcaccgtgagctcagcggccgcgctgagcaacagcatcatgtacttcagccacttcgtgcctgtgttcctgcctgccaagcctacaacaacaccagcccctagacctccaacccctgcccctacaattgcctctcagcctctgtctctgaggcccgaagcttgtagacctgctgctggcggagctgtgcacaccagaggactggatttcgcctgcttttgggtgctggtggtcgtgggcggagtgctggcttgttattctctgctggtcaccgtggccttcatcatcttttgggtccgactgaagatccaggtccgaaaggccgccatcaccagctacgagaagtctgatggcgtgtacaccggcctgagcaccagaaaccaggaaacctacgagacactgaagcacgagaagcccccccag

SEQ ID NO: 69 - protein, 405 aa, synthetic construct
  REGION 1..405: note = Laboratory made
MDWIWRILFLVGAATGAHSAQPANIQMTQSPSSVSASVGDRVTITCRASQDISRWLAWYQQKPGKAPKLLIYAASSLQSGVPSRFSGSGSGTDFALTISSLQPEDFATYYCQQADSRFSITFGQGTRLEIKGGGGSGGGGSGGGGSGGGGSEVQLVQSGGGLVQPGGSLRLSCAASGFTFSSYSMNWVRQAPGKGLEWVSYISSSSSTIQYADSVKGRFTISRDNAKNSLYLQMNSLRDEDTAVYYCARGDYYYGMDVWGQGTTVTVSSAAALSNSIMYFSHFVPVFLPAKPTTTPAPRPPTPAPTIASQPLSLRPEACRPAAGGAVHTRGLDFACFWVLVVVGGVLACYSLLVTVAFIIFWVRLKIQVRKAAITSYEKSDGVYTGLSTRNQETYETLKHEKPPQ